European Patent Application EP 4 717 703 A1, published April 1, 2026. Title: A CEA-binding polypeptide. Applicant: Zytox Therapeutics AB. Application EP. The sequence listing filed with the application follows.

SEQUENCE LISTING (59 sequences)

SEQ ID NO: 1 - skipped

SEQ ID NO: 2 - protein, 5 aa, synthetic construct
WWFAW

SEQ ID NO: 3 - protein, 5 aa, synthetic construct
WWKAY

SEQ ID NO: 4 - protein, 5 aa, synthetic construct
WWHAY

SEQ ID NO: 5 - protein, 5 aa, synthetic construct
WWYAY

SEQ ID NO: 6 - protein, 5 aa, synthetic construct
WWDAY

SEQ ID NO: 7 - protein, 5 aa, synthetic construct
FWVAY

SEQ ID NO: 8 - protein, 5 aa, synthetic construct
FWFAY

SEQ ID NO: 9 - protein, 5 aa, synthetic construct
WWAAW

SEQ ID NO: 10 - protein, 5 aa, synthetic construct
WWGAY

SEQ ID NO: 11 - protein, 5 aa, synthetic construct
FWNAW

SEQ ID NO: 12 - protein, 5 aa, synthetic construct
FWEAY

SEQ ID NO: 13 - protein, 5 aa, synthetic construct
WWAFY

SEQ ID NO: 14 - protein, 5 aa, synthetic construct
FWAFY

SEQ ID NO: 15 - protein, 27 aa, synthetic construct
WWHAYHEIHDLPNLNIKQRKAFIFSLM

SEQ ID NO: 16 - protein, 27 aa, synthetic construct
WWYAYSEIHSLPNLNDRQHHAFIASLI

SEQ ID NO: 17 - protein, 27 aa, synthetic construct
WWDAYHEIRILPNLNSEQTVAFIKSLM

SEQ ID NO: 18 - protein, 27 aa, synthetic construct
FWVAYHEIRELPNLNTTQTRAFIRSLS

SEQ ID NO: 19 - protein, 27 aa, synthetic construct
WWFAWSEIVNLPNLNKDQQVAFKHSLV

SEQ ID NO: 20 - protein, 27 aa, synthetic construct
WWKAYAEIITLPNLNRNQSSAFIRSLV

SEQ ID NO: 21 - protein, 27 aa, synthetic construct
WWHAYHEIMTLPNLNRIQQHAFIQSLM

SEQ ID NO: 22 - protein, 27 aa, synthetic construct
WWKAYHEIRDLPNLNAEQRGAFIQSLM

SEQ ID NO: 23 - protein, 27 aa, synthetic construct
WWKAYHEIRTLPNLNVEQETAFIRSLA

SEQ ID NO: 24 - protein, 27 aa, synthetic construct
FWFAYHEIRVLPNLNAGQSHAFIQSLT

SEQ ID NO: 25 - protein, 27 aa, synthetic construct
WWHAYHEIHDLPNLNDAQIMAFKKSLM

SEQ ID NO: 26 - protein, 27 aa, synthetic construct
WWHAYHEIKDLPNLNEGQLSAFIRSLM

SEQ ID NO: 27 - protein, 27 aa, synthetic construct
WWGAYHEIRELPNLNDEQVHAFIRSLM

SEQ ID NO: 28 - protein, 27 aa, synthetic construct
WWAAWSEIMVLPNLNMQQRQAFKQSLV

SEQ ID NO: 29 - protein, 27 aa, synthetic construct
FWNAWHEIRVLPNLNQFQTDAFILSLM

SEQ ID NO: 30 - protein, 27 aa, synthetic construct
FWEAYHEIITLPNLNKEQNIAFIRSLL

SEQ ID NO: 31 - protein, 27 aa, synthetic construct
WWYAYHEIIHLPNLNIGQTKAFIRSLV

SEQ ID NO: 32 - protein, 27 aa, synthetic construct
QVMAIKEIIKLPNLNANQWWAFYHSLY

SEQ ID NO: 33 - protein, 27 aa, synthetic construct
MQAATREIMSLPNLNGQQFWAFYHSLR

SEQ ID NO: 34 - protein, 58 aa, synthetic construct
VDNKFNKEWWHAYHEIHDLPNLNIKQRKAFIFSLMDDPSQSANLLAEAKKLNDAQAPK

SEQ ID NO: 35 - protein, 58 aa, synthetic construct
VDNKFNKEWWYAYSEIHSLPNLNDRQHHAFIASLIDDPSQSANLLAEAKKLNDAQAPK

SEQ ID NO: 36 - protein, 58 aa, synthetic construct
VDNKFNKEWWDAYHEIRILPNLNSEQTVAFIKSLMDDPSQSANLLAEAKKLNDAQAPK

SEQ ID NO: 37 - protein, 58 aa, synthetic construct
VDNKFNKEFWVAYHEIRELPNLNTTQTRAFIRSLSDDPSQSANLLAEAKKLNDAQAPK

SEQ ID NO: 38 - protein, 58 aa, synthetic construct
VDNKFNKEWWFAWSEIVNLPNLNKDQQVAFKHSLVDDPSQSANLLAEAKKLNDAQAPK

SEQ ID NO: 39 - protein, 58 aa, synthetic construct
VDNKFNKEWWKAYAEIITLPNLNRNQSSAFIRSLVDDPSQSANLLAEAKKLNDAQAPK

SEQ ID NO: 40 - protein, 58 aa, synthetic construct
VDNKFNKEWWHAYHEIMTLPNLNRIQQHAFIQSLMDDPSQSANLLAEAKKLNDAQAPK

SEQ ID NO: 41 - protein, 58 aa, synthetic construct
VDNKFNKEWWKAYHEIRDLPNLNAEQRGAFIQSLMDDPSQSANLLAEAKKLNDAQAPK

SEQ ID NO: 42 - protein, 58 aa, synthetic construct
VDNKFNKEWWKAYHEIRTLPNLNVEQETAFIRSLADDPSQSANLLAEAKKLNDAQAPK

SEQ ID NO: 43 - protein, 58 aa, synthetic construct
VDNKFNKEFWFAYHEIRVLPNLNAGQSHAFIQSLTDDPSQSANLLAEAKKLNDAQAPK

SEQ ID NO: 44 - protein, 58 aa, synthetic construct
VDNKFNKEWWHAYHEIHDLPNLNDAQIMAFKKSLMDDPSQSANLLAEAKKLNDAQAPK

SEQ ID NO: 45 - protein, 58 aa, synthetic construct
VDNKFNKEWWHAYHEIKDLPNLNEGQLSAFIRSLMDDPSQSANLLAEAKKLNDAQAPK

SEQ ID NO: 46 - protein, 58 aa, synthetic construct
VDNKFNKEWWGAYHEIRELPNLNDEQVHAFIRSLMDDPSQSANLLAEAKKLNDAQAPK

SEQ ID NO: 47 - protein, 58 aa, synthetic construct
VDNKFNKEWWAAWSEIMVLPNLNMQQRQAFKQSLVDDPSQSANLLAEAKKLNDAQAPK

SEQ ID NO: 48 - protein, 58 aa, synthetic construct
VDNKFNKEFWNAWHEIRVLPNLNQFQTDAFILSLMDDPSQSANLLAEAKKLNDAQAPK

SEQ ID NO: 49 - protein, 58 aa, synthetic construct
VDNKFNKEFWEAYHEIITLPNLNKEQNIAFIRSLLDDPSQSANLLAEAKKLNDAQAPK

SEQ ID NO: 50 - protein, 58 aa, synthetic construct
VDNKFNKEWWYAYHEIIHLPNLNIGQTKAFIRSLVDDPSQSANLLAEAKKLNDAQTPK

SEQ ID NO: 51 - protein, 58 aa, synthetic construct
VDNKFNKEQVMAIKEIIKLPNLNANQWWAFYHSLYDDPSQSANLLAEAKKLNDAQAPK

SEQ ID NO: 52 - protein, 58 aa, synthetic construct
VDNKFNKEMQAATREIMSLPNLNGQQFWAFYHSLRDDPSQSANLLAEAKKLNDAQAPK

SEQ ID NO: 53-54 - skipped (2 entries)

SEQ ID NO: 55 - protein, 13 aa, synthetic construct
ANLLAEAKKLNDA

SEQ ID NO: 56 - protein, 13 aa, synthetic construct
SELLSEAKKLNDS

SEQ ID NO: 57 - protein, 6 aa, synthetic construct
GARRAG

SEQ ID NO: 58 - protein, 4 aa, synthetic construct
GRGA

SEQ ID NO: 59 - protein, 5 aa, synthetic construct
GGGSG